European Patent Application EP 4 451 275 A1, published October 23, 2024. Title: METHODS AND SYSTEMS FOR PREDICTING A CATEGORY OF MAMMOGRAPHIC BREAST DENSITY FOR A SUBJECT. Applicant: Tata Consultancy Services Limited. Application EP. The sequence listing filed with the application follows.

SEQUENCE LISTING (13 sequences)

SEQ ID NO: 1 - RNA, 1433 nt, Murimonas intestini strain SRB-530-5-H
  source 1..1433: mol_type = rRNA
tgcagtcgagcggagtatttaacggaagtcttcggatggaagtttggatacttagcggcggacgggtgagtaacgcgtgggcaacctgccccataccgggggataacagccagaaatggctgctaataccgcataagcgcacagcgccacatggcgcggtgtgaaaaactccggtggtatgggatgggcccgcgtctgattaggtagttggcggggtaacggcccaccaagccgacgatcagtagccgacctgagagggtgaccggccacattgggactgagacacggcccaaactcctacgggaggcagcagtggggaatattgcacaatgggggaaaccctgatgcagcgacgccgcgtgagcgaagaagtatttcggtatgtaaagctctatcagcagggaagaaaatgacggtacctgactaagaagccccggctaactacgtgccagcagccgcggtaatacgtagggggcaagcgttatccggatttactgggtgtaaagggagcgtagacggccaggcaagtctgatgtgaaaggcaggggctcaacccctggactgcattggaaactgtcaggctggagtgccggagaggtaagcggaattcctagtgtagcggtgaaatgcgtagatattaggaggaacaccagtggcgaaggcggcttactggacggtaactgacgttgatgctcgaaagcgtggggagcaaacaggattagataccctggtagtccacgccgtaaacgatgaatactaggtgtcggggggcaaagcccttcggtgccgccgcaaacgcattaagtattccacctggggagtacgttcgcaagaatgaaactcaaaggaattgacggggacccgcacaagcggtggagcatgtggtttaattcgaagcaacgcgaagaaccttaccaagccttgacatcccattgaagccagagtaacgtctgacggccttcgggacaatggagacaggtggtgcatggttgtcgtcagctcgtgtcgtgagatgttgggttaagtcccgcaacgagcgcaacccttatcttcagtagccagcacgcgatggtgggcactctggagagactgccagggacaacctggaggaaggtggggatgacgtcaaatcatcatgccccttatggcttgggctacacacgtgctacaatggcgtaaacagagggaagcagccctgcgaaggtgagcgaatcccaaaaataacgtctcagttcggattgtagtctgcaactcgactacatgaagctggaatcgctagtaatcgcgaatcagaatgtcgcggtgaatacgttcccgggtcttgtacacaccgcccgtcacaccatgggagtcagtaacgcccgaagtcagtgacctaaaccgaaaggaaggagctgccgaaggcgggactggtaactggggtgaagtcgtaa

SEQ ID NO: 2 - RNA, 1394 nt, Clostridium perfringens strain A
  source 1..1394: mol_type = rRNA
atgcaagtcgtaacaaggtagccgttatagggaacggattagcggcggacgggtgagtaacacgtgggtaacctgcctcatagagtggaatagccttccgaaaggaagattaataccgcataatgttgaaagatggcatcatcattcaaccaaaggagcaatccgctatgagatggacccgcggcgcattagctagttggtggggtaacggcctaccaaggcgacgatgcgtagccgacctgagagggtgatcggccacattgggactgagacacggcccagactcctacgggaggcagcagtggggaatattgcacaatgggggaaaccctgatgcagcaacgccgcgtgagtgatgaaggttttcggatcgtaaagctctgtctttggggaagataatgacggtacccaaggaggaagccacggctaactacgtgccagcagccgcggtaatacgtaggtggcgagcgttatccggatttactgggcgtaaagggagcgtaggcggatgatkwrgkggratgtgaaatagcccggkctcaacttgggtgctgcattaccaaactsgttatctagagtgcaggagaggagagtrgaattcstagtgtagcggtgaaatgcgtakagattakgaagaacaccagtggcgaaggcgactctctggactgtaactgacgctgaggctcgaaagcgtggggagcaaacaggattagataccctggtagtccacgccgtawacgatgaatactaggtgtggggggtttcaacacctccgtgccgccgctaacgcattwagtattccgtcctggrgaagtacggtcgcarrattamaactcraaggaatttgacggggasctcgcaacaaagttagcggagcatgtsgtttaattcgaagcaacgcgaagaaccttacctacacttgacatcccttgcattactcttaatcgaggaaatcccttcggggacaaggtgacaggtggtgcatggttgtcgtcagctcgtgtcgtgagatgttgggttaagtcccgcaacgagcgcaacccttgtcgttagttactaccattaagttgaggactctagcgagactgcctgggttaaccaggaggaaggtggggatgacgtcaaatcatcatgccccttatgtgtagggctacacacgtgctacaatggctggtacagagagatgcaataccgcgaggtggagcctaacttaaaaaccagtctcagttcggattgtaggctgaaactcgcctacatgaagctggagttactagtaatcgcgaatcagaatgtcgcggtgaatacgttcccgggtcttgtacacaccgcccgtcacaccatgagagttggcaatacccgaagttcgtagagtttgatccctggctcagataacg

SEQ ID NO: 3 - RNA, 1481 nt, [Ruminococcus] gnavus ATCC 29149
  source 1..1481: mol_type = rRNA
tgaacgctggcggcgtgcttaacacatgcaagtcgagcgaagcaccttgacggatttcttcggattgaagccttggtgactgagcggcggacgggtgagtaacgcgtgggtaacctgcctcatacagggggataacagttggaaacgnctgctaataccgcataagcgcacagtaccgcatggtacggtgtgaaaaactccggtggtatgagatggacccgcgtctgattaggtagttggtggggtaacggcctaccaagccgacgatcagtagccgacctgagagggtgaccggccacattgggactgagacacggcccaaactcctacgggaggcagcagtggggaatattgcacaatgggggaaaccctgatgcagcgacgccgcgtgagcgatgaagtatttcggtatgtaaagctctatcagcagggaagaaaatgacggtacctgactaagaagccccggctaactacgtgccagcagccgcggtaatacgtagggggcaagcgttatccggatttactgggtgtaaagggagcgtagacggcatggcaagccagatgtgaaagcccggggctcaaccccgggactgcatttggaactgtcaggctagagtgtcggagaggaaagcggaattcctagtgtagcggtgaaatgcgtagatattaggaggaacaccagtggcgaaggcggctttctggacgatgactgacgttgaggctcgaaagcgtggggagcaaacaggattagataccctggtagtccacgccgtaaacgatgaatactaggtgtcgggtggcaaagccattcggtgccgcagcaaacgcaataagtattccacctggggagtacgttcgcaagaatgaaactcaaaggaattgacggggacccgcacaagcggtggagcatgtggtttaattcgaagcaacgcgaagaaccttacctggtcttgacatccctctgaccgctctttaatcggagctttccttcgggacagaggagacaggtggtgcatggttgtcgtcagctcgtgtcgtgagatgttgggttaagtcccgcaacgagcgcancccctatctttagtagccagcattttggatgggcactctagagagactgccagggataacctggaggaaggtggggatgacgtcaaatcatcatgccccttatgaccagggctacacacgtgctacaatggcgtaaacaaagggaagcgagcccgcgagggggagcaaatcccaaaaataacgtctcagttcggattgtagtctgcaactcgactacatgaagctggaatcgctagtaatcgcgaatcagaatgtcgcggtgaatacgtncccgggtcttgtacacaccgcccgtcacaccatgggagtcagtaacgcccgaagtcagtgacccaaccgcaaggagggagctgccgaaggtgggaccgataactggggtgaagtcgtaacaaggtagccgtatcggaagg

SEQ ID NO: 4 - RNA, 1440 nt, Coprococcus eutactus strain ATCC 27759
  source 1..1440: mol_type = rRNA
gatgaacgctggcggcgtgcttaacacatgcaagtcgaacgattgaagctggagcttgctccggccgatttagtggcggacgggtgagtaacgcgtgggtaacctgcctcatacagggggatagcagttggaaacgactggtaaaaccgcataagcgcacrgtatcgcatgatacagtgtgaaaacactccggtggtatgagatggacccgcgtctgattagctagttggtgaggtaacggcccaccaaggcgacgatcagtagccggcctgagagggtgaacggccacattgggactgagacacggcccaaactcctacgggaggcagcagtggggaatattgcacaatgggggaaaccctgatgcagcgacgccgcgtgagtgaagaagtatttcggtatgtaaagctctatcagcagggaagataatgacggtacctgactaagaagcaccggctaaatacgtgccagcagccgcggtaatacgtatggtgcaagcgttatccggatttactgggtgtaaagggtgcgtaggtggcaaggcaagtctgaagtgaaaatccggggctcaaccccggaactgctttggaaactgtttagctagagtacaggagaggtaagtggaattcctagtgtagcggtgaaatgcgtagatattaggaggaacaccagtggcgaaggcgacttactggactgctactgacactgaggcacgaaagcgtggggagcaaacaggattagataccctggtagtccacgccgtaaacgatgaatactaggtgttgggttccaaagggactcggtgccgtcgcaaacgcattaagtattccacctggggagtacgttcgcaagaatgaaactcaaaggaattgacggggacccgcacaagcggtggagcatgtggtttaattcgaagcaacgcgaaaaaccttaccaagtcttgacatcctgatgacggttccttaaccggaacttctcttcggagcatcagagacaggtggtgcatggttgtcgtcagctcgtgtcgtgagatgttgggttaagtcccgcaacgagcgcaacccctatttccagtagccagcagtaagatgggcactctggagagactgccggggataacccggaggaaggtggggatgacgtcaaatcatcatgccccttatgatttgggctacacacgtgctacaatggcagttacaaagagaagcraacctgtgaaggcgagcaaacctcaaaaaggctgtctcagttcggattgtagtctgcaactcgactacatgaagctggaatcgctagtaatcgcagatcagcatgctgcggtgaatacgttcccgggtcttgtacacaccgcccgtcacaccatgggagtcggtaacgcccgaagtcagtgacccaaccgcaaggagggagctgccgaaggcaggatcgataactggggtg

SEQ ID NO: 5 - RNA, 1521 nt, [Eubacterium] rectale ATCC 33656
  source 1..1521: mol_type = rRNA
agagtttgatcctggctcaggatgaacgctggcggcgtgcttaacacatgcaagtcgaacgaagcactttatttgatttccttcgggactgattattttgtgactgagtggcggacgggtgagtaacgcgtgggtaacctgccttgtacagggggataacagttggaaacggctgctaataccgcataagcgcacggcatcgcatgatgcagtgtgaaaaactccggtggtataagatggacccgcgttggattagctagttggtgaggtaacggcccaccaaggcgacgatccatagccgacctgagagggtgaccggccacattgggactgagacacggcccaaactcctacgggaggcagcagtggggaatattgcacaatgggcgaaagcctgatgcagcgacgccgcgtgagcgaagaagtatttcggtatgtaaagctctatcagcagggaagataatgacggtacctgactaagaagcaccggctaaatacgtgccagcagccgcggtaatacgtatggtgcaagcgttatccggatttactgggtgtaaagggagcgcaggcggtgcggcaagtctgatgtgaaagcccggggctcaaccccggtactgcattggaaactgtcgtactagagtgtcggaggggtaagcggaattcctagtgtagcggtgaaatgcgtagatattaggaggaacaccagtggcgaaggcggcttactggacgataactgacgctgaggctcgaaagcgtggggagcaaacaggattagataccctggtagtccacgccgtaaacgatgaatactaggtgttgggaagcattgcttctcggtgccgtcgcaaacgcagtaagtattccacctggggagtacgttcgcaagaatgaaactcaaaggaattgacggggacccgcacaagcggtggagcatgtggtttaattcgaagcaacgcgaagaaccttaccaagtcttgacatccttctgaccggtacttaaccgtaccttctcttcggagcaggagtgacaggtggtgcatggttgtcgtcagctcgtgtcgtgagatgttgggttaagtcccgcaacgagcgcaacccttatctttagtagccagcggttcggccgggcactctagagagactgccagggataacctggaggaaggcggggatgacgtcaaatcatcatgccccttatgacttgggctacacacgtgctacaatggcgtaaacaaagggaagcaaagctgtgaagccgagcaaatctcaaaaataacgtctcagttcggactgtagtctgcaacccgactacacgaagctggaatcgctagtaatcgcagatcagaatgctgcggtgaatacgttcccgggtcttgtacacaccgcccgtcacaccatgggagttgggaatgcccgaagccagtgacctaaccgaaaggaaggagctgtcgaaggcaggctcgataactggggtgaagtcgtaacaaggtagccgtatcggaaggtgcggctggatcacct

SEQ ID NO: 6 - RNA, 1492 nt, Blautia hansenii DSM 20583 strain JCM 14655
  source 1..1492: mol_type = rRNA
agagtttgatcctggctcaggatgaacgctggcggcgtgcttaacacatgcaagtcgagcgaagcacttatcattgactcttcggaagatttgatatttgactgagcggcggacgggtgagtaacgcgtgggtaacctgcctcatacaggggaataacagttagaaatggctgctaatgccgcataagcgcacaggaccgcatggtctggtgtgaaaaactgaggtggtatgagatggacccgcgtctgattaggtagttggtggggtaacggcctaccaagccgacgatcagtagccggcctgagagggtgaacggccacattgggactgagacacggcccagactcctacgggaggcagcagtggggaatattgcacaatgggggaaaccctgatgcagcgacgccgcgtgaaggaagaagtatctcggtatgtaaacttctatcagcagggaagaaaatgacggtacctgactaagaagccccggctaactacgtgccagcagccgcggtaatacgtagggggcaagcgttatccggatttactgggtgtaaagggagcgtagacggaagagcaagtctgatgtgaaaggctggggcttaaccccaggactgcattggaaactgtttttctagagtgccggagaggtaagcggaattcctagtgtagcggtgaaatgcgtagatattaggaggaacaccagtggcgaaggcggcttactggacggtaactgacgttgaggctcgaaagcgtggggagcaaacaggattagataccctggtagtccacgccgtaaacgatgaatactaggtgtcggggtgcaaagcagttcggtgccgcagcaaacgcaataagtattccacctggggagtacgttcgcaagaatgaaactcaaaggaattgacggggacccgcacaagcggtggagcatgtggtttaattcgaagcaacgcgaagaaccttaccaagtcttgacatctgcctgaccgttccttaaccggagctttccttcgggacaggcaagacaggtggtgcatggttgtcgtcagctcgtgtcgtgagatgttgggttaagtcccgcaacgagcgcaacccctatccttagtagccagcagtccggctgggcactctagggagactgccggggataacccggaggaaggcggggacgacgtcaaatcatcatgccccttatgatttgggctacacacgtgctacaatggcgtaaacaaagggaagcgaagcggtgacgcttagcaaatctcaaaaataacgtcccagttcggactgcagtctgcaactcgactgcacgaagctggaatcgctagtaatcgcgaatcagaatgtcgcggtgaatacgttcccgggtcttgtacacaccgcccgtcacaccatgggagtcagtaacgcccgaagtcagtgacccaaccttatggagggagctgccgaaggcgggaccgataactggggtgaagtcgtaacaaggtaacc

SEQ ID NO: 7 - RNA, 1262 nt, Blautia faecis strain M25
  source 1..1262: mol_type = rRNA
ataacagccagaaatgactgctaataccgcataagcgcacagaaccgcatggttcggtgtgaaaaactccggtggtataagatggacccgcgttggattagctagttggcagggcagcggcctaccaaggcgacgatccatagccggcctgagagggtgaacggccacattgggactgagacacggcccagactcctacgggaggcagcagtggggaatattgcacaatgggggaaaccctgatgcagcgacgccgcgtgaaggaagaagtatctcggtatgtaaacttctatcagcagggaagataatgacggtacctgactaagaagccccggctaactacgtgccagcagccgcggtaatacgtagggggcaagcgttatccggatttactgggtgtaaagggagcgtagacggcgcagcaagtctgatgtgaaaggcaggggcttaacccctggactgcattggaaactgctgtgcttgagtgccggaggggtaagcggaattcctagtgtagcggtgaaatgcgtagatattaggaggaacaccagtggcgaaggcggcttactggacggtaactgacgttgaggctcgaaagcgtggggagcaaacaggattagataccctggtagtccacgccgtaaacgatgaatactaggtgtcagggagcacagctctttggtgccgccgcaaacgcattaagtattccacctggggagtacgttcgcaagaatgaaactcaaaggaattgacggggacccgcacaagcggtggagcatgtggtttaattcgaagcaacgcgaagaaccttaccaaatcttgacatccctctgaccgggacttaaccgtccctttccttcgggacaggggagacaggtggtgcatggttgtcgtcagctcgtgtcgtgagatgttgggttaagtcccgcaacgagcgcaacccctatccttagtagccagcacgcartggtgggcactctgaggagactgccagggataacctggaggaaggcggggatgacgtcaaatcatcatgccccttatgatttgggctacacacgtgctacaatggcgtaaacaaagggaagcgaacccgcgagggtgggcaaatctcaaaaataacgtcccagttcggactgcagtctgcaactcgactgcacgaagctggaatcgctagtaatcgcggatcagaatgccgcggtgaatacgttcccgggtcttgtacacaccgcccgtcacaccatgggagtcagtaacgcccg

SEQ ID NO: 8 - RNA, 1378 nt, Blautia caecimuris strain SJ18
  source 1..1378: mol_type = rRNA
attttgacagagacttcggttgaagtcgttataatcctagtggcggacgggtgagtaacgcgtgggtaacctgcctcacactgggggataacagtcagaaatgactgctaataccgcataagcgcacgggattgcatgatccagtgtgaaaaactccggtggtgtgagatggacccgcgttggattagccagttggcagggtaacggcctaccaaagcgacgatccatagccggcctgagagggtggacggccacattgggactgagacacggcccagactcctacgggaggcagcagtggggaatattgcacaatgggggaaaccctgatgcagcgacgccgcgtgaaggaagaagtatctcggtatgtaaacttctatcagcagggaagaaaatgacggtacctgactaaaaagccccggctaactacgtgccagcagccgcggtaatacgtagggggcaagcgttatccggatttactgggtgtaaagggagcgtagacggagcagcaagtctgatgtgaaaggcgggggctcaacccccggactgcattggaaactgttgatcttgagtaccggagaggtaagcggaattcctagtgtagcggtgaaatgcgtagatattaggaggaacaccagtggcgaaggcggcttactggacggtaactgacgttgaggctcgaaagcgtggggagcaaacaggattagataccctggtagtccacgccgtaaacgatgaatactaggtgtcgggtggcagagccattcggtgccgcagcaaacgcagtaagtattccacctgggggagtacgttcgcaagaatgaaactcaaaggaattgacggggacccgcacaagcggtggagcatgtggtttaattcgaagcaacgcgaagaaccttaccaagtcttgacatccctatgaccggcgcgtaacgtcgccttttcttcggagcatcggagacaggtggtgcatggttgtcgtcagctcgtgtcgtgagatgttgggttaagtcccgcaacgagcgcaacccctatccttagtagccagcggtttggccgggcactctgaggagactgccagggataacctggaggaaggcggggatgacgtcaaatcatcatgccccttatgatttgggctacacacgtgctacaatggcgtaaacaaagggaagcgagagtgtgagcttaagcaaatcccaaaaataacgtcccagttcggactgcagtctgcaactcgactgcacgaagctggaatcgctagtaatcgcggatcagaatgccgcggtgaatacgttcccgggtcttgtacacaccgcccgtcacaccatgggagtcagtaacgcccgaagtcaggaccgaaccgaaaggacggagc

SEQ ID NO: 9 - RNA, 1476 nt, Bacteroides vulgatus
  source 1..1476: mol_type = rRNA
caaactaggaccgagtcctacttgcgatcgatgtccgaattgtgtacgttcagctccccgtcgtaccagaatcgaacgattccggctaccgctggccgcgtgcccactcattgtgcataggttggacggcagatgagaacctgtcggaagactttccttctaattatgttctaccgtagtactcaggcgtacaagtgtactaatttccataaggccatctgctacccctacgcaaggtaatctatcatccgccccattgccgggtggatcagaagctacctatcccaagactctccttcagggggtgtaaccttgactctgtgccaggtttgaggatgccctccgtcgtcactccttataaccagttacccgctctcggacttggtcggttcatcgcacttcctactgacgggatacccaacatttgaagaaaatatttccttatttcagcccatacctatgggcaaacgtacatgaaatacttattcctagccgattgaggcacggtcgtcggcgccattatgcctcctaggctcgcaataggcctaaataacccaaatttccctcgcatctacctacaaattcagtcaacactttcaaacgccgagttggcattttaacgtcaactatgacctatagaactcacgtcaactccgtccgccttaagcaccacatcgccactttacgaatctatagtgcttcttgaggctaacgcttccgtcggacgattcgacgttgactgtaactccgagctttcacacccatagtttgtcctaatctatgggaccatcaggtgtgccatttgctacttatgagcgacaaacgctatatgccgttcgccggttcgctttcgcaattcataaggtggacccctcatgcggccgttgccactttgagtttccttaactgcccccgggcgtgttcgcctccttgtacaccaaattaagctactatgcgctccttggaatgggcccgaatttaacgtctacttaatgccactttcggcattcggcgttccgtagacacttccacgacgtaccaacagcagtcgagcacggcactccacagccgaattcacggtattgctcgcgttgggaacaacagtcaatgattgtccaaaacgactcctgagactgttctgacggtagcattctacactccttccacccctactgcagtttagtcgtgccgggaatgcaggccccgatgtgtgcacaatgttaccccccatgtctcccggcgatggtgcgctcactacggttaggggttttggagagagtcaagcctgacctcagacgttgggctgaggtgcttcgacctaagcgatcattagcgcgtagtcggtgccgcgccacttatgcaagggcccggaacatgtgtggcgggcagttcggtaccctcggccccccatggacttcacgcattggcgctcctcgcgggatcccattttgaccactgaccccgattcagcattgt

SEQ ID NO: 10 - RNA, 1455 nt, Bacteroides ovatus strain JCM 5824
  source 1..1455: mol_type = rRNA
gatcatggctcaggatgaacgctagctacaggcttaacacatacaagtcgtggggcagcattttatgtttgtttgcaaactgaagatggcgaccggcgcacgggtgagtaacacgtatccaacctgccgataactccggaatagcctttcgaaagaaagattaataccggatagcatacgatatcgcatgatatttttattaaagaatttcggttatcgatggggatgcgttccattagtttgttggcggggtaacggcccaccaagactacgatggataggggttctgagaggaaggtcccccacattggaactgagacacggtccaaactcctacgggaggcagcagtgaggaatattggtcaatgggcgagagcctgaaccagccaagtagcgtgaaggatgaaggctctatgggtcgtaaacttcttttatatgggaataaagttttccacgtgtggaattttgtatgtaccatatgaataaggatcggactactccgtgccagcagccgcggtaatacggaggatccgagcgttatccggatttattgggtttaaagggagcgtaggtggattgttaagtcagttgtgaaagtttgcggctcaaccgtaaaattgcagttgaaactggcagtcttgagtacagtagaggtgggcggaattcgtggtgtagcggtgaaatgcttagatatcacgaagaactccgattgcgaaggcagctcactagactgttactgacactgatgctcgaaagtgtgggtatcaaacaggattagataccctggtagtccacacagtaaacgatgaatactcgctgtttgcgatatacagtaagcggccaagcgaaagcattaagtattccacctggggagtacgccggcaacggtgaaactcaaaggaattgacgggggcccgcacaagcggaggaacatgtggtttaattcgatgatacgcgagaaccttacccgggcttaaattgcaacagaatatattggaaacagtatagccgtaaggctgttgtgaaggtgctgcatggttgtcgtcagctcgtgccgtgaggtgtcggcttaagtgccataacgagcgcaacccttatctttagttactaacaggttatgctgaggactctagagagactgccgtcgtaagatgtgaggaaggtggggatgacgtcaaatcagcacggcccttacgtccggggctacacacgtgttacaatggggggtacagaaggcagctacctggtgacatgatgctaatcccaaaaacctctctcagttcggatcgaagtctgcaacccgacttcgtgaagctggattcgctagtaatcgcgcatcagccatggcgcggtgaatacgttcccgggccttgtacacaccgcccgtcaagccatgaaagccgggggtacctgaagtacgtaaccgcaaggagcgtcctagggtaaaactggtaa

SEQ ID NO: 11 - RNA, 1529 nt, Bacteroides fragilis NCTC 9343
  source 1..1529: mol_type = rRNA
acaatgaagagtttgatcctggctcaggatgaacgctagctacaggcttaacacatgcaagtcgaggggcatcaggaagaaagcttgctttctttgctggcgaccggcgcacgggtgagtaacacgtatccaacctgccctttactcggggatagcctttcgaaagaaagattaatacccgatagcataatgattccgcatggtttcattattaaaggattccggtaaaggatggggatgcgttccattaggttgttggtgaggtaacggctcaccaagccttcgatggataggggttctgagaggaaggtcccccacattggaactgagacacggtccaaactcctacgggaggcagcagtgaggaatattggtcaatgggcgctagcctgaaccagccaagtagcgtgaaggatgaaggctctatgggtcgtaaacttcttttatataagaataaagtgcagtatgtatactgttttgtatgtattatatgaataaggatcggctaactccgtgccagcagccgcggtaatacggaggatccgagcgttatccggatttattgggtttaaagggagcgtaggtggactggtaagtcagttgtgaaagtttgcggctcaaccgtaaaattgcagttgatactgtcagtcttgagtacagtagaggtgggcggaattcgtggtgtagcggtgaaatgcttagatatcacgaagaactccgattgcgaaggcagctcactggactgcaactgacactgatgctcgaaagtgtgggtatcaaacaggattagataccctggtagtccacacagtaaacgatgaatactcgctgtttgcgatatacagtaagcggccaagcgaaagcattaagtattccacctggggagtacgccggcaacggtgaaactcaaaggaattgacgggggcccgcacaagcggaggaacatgtggtttaattcgatgatacgcgaggaaccttacccgggcttaaattgcagtggaatgatgtggaaacatgtcagtgagcaatcaccgctgtgaaggtgctgcatggttgtcgtcagctcgtgccgtgaggtgtcggcttaagtgccataacgagcgcaacccttatctttagttactaacaggttatgctgaggactctagagagactgccgtcgtaagatgtgaggaaggtggggatgacgtcaaatcagcacggcccttacgtccggggctacacacgtgttacaatggggggtacagaaggcagctagcgggtgaccgtatgctaatcccaaaatcctctctcagttcggatcgaagtctgcaacccgacttcgtgaagctggattcgctagtaatcgcgcatcagccacggcgcggtgaatacgttcccgggccttgtacacaccgcccgtcaagccatgggagccgggggtacctgaagtacgtaaccgcaaggatcgtcctagggtaaaactggtgactggggctaagtcgtaacaaggtagccgtaccggaaggtgcggctggaacacctccttt

SEQ ID NO: 12 - RNA, 1429 nt, Intestinibacter bartlettii strain WAL 16138
  source 1..1429: mol_type = rRNA
aggatgaacgctggcggcgtgcctaacacatgcaagtcgagcgattntcttcggagaagagcggcggacgggtgagtaacgcgtgggtaacctgccctgtacacacggataacataccgaaaggtatgctaatacgggataacataagaaattcgcatgtttttcttatcaaagctccggcggtacaggatggacccgcgtctgattagctagttggtgaggtaacggctcaccaaggcgacgatcagtagccgacctgagagggtgatcggccacattggaactgagacacggtccaaactcctacgggaggcagcagtggggaatattgcacaatgggcgaaagcctgatgcagcaacgccgcgtgagcgatgaaggccttcgggtcgtaaagctctgtcctcaaggaagataatgacggtacttgaggaggaagccccggctaactacgtgccagcagccgcggtaatacgtagggggctagcgttatccggatttactgggcgtaaagggtgcgtaggcggtcttttaagtcaggagtgaaaggctacggctcaaccgtagtaagctcttgaaactggaggacttgagtgcaggagaggagagtggaattcctagtgtagcggtgaaatgcgtagatattaggaggaacaccagtagcgaaggcggctctctggactgtaactgacgctgaggcacgaaagcgtggggagcaaacaggattagataccctggtagtccacgccgtaaacgatgagtactagctgtcggaggttacccccttcggtggcgcagctaacgcattaagtactccgcctggggagtacgctcgcaagagtgaaactcaaaggaattgacggggacccgcacaagtagcggagcatgtggtttaattcgaagcaacgcgaagaaccttacctaagcttgacatccttttgaccgatgcctaatcgcatctttcccttcggggacagaagtgacaggtggtgcatggttgtcgtcagctcgtgtcgtgagatgttgggttaagtcccgcaacgagcgcaacccttgcctttagttgccatcattaagttgggcactctagagggactgccagggataacctggaggaaggtggggatgacgtcaaatcatcatgccccttatgcttagggctacacacgtgctacaatgggtggtacagagggcagcgaagtcgtgaggccaagctaatcccttaaagccattctcagttcggattgtaggctgaaactcgcctacatgaagctggagttactagtaatcgcagatcagaatgctgcggtgaatgcgttcccgggtcttgtacacaccgcccgtcacaccatgggagttgggggcgcccgaagccggctagctaaccttttggaagcggtcgtcgaaggtgaaaccaataactggggtgaa

SEQ ID NO: 13 - RNA, 1454 nt, Bilophila wadsworthia strain CCUG 32349
  source 1..1454: mol_type = rRNA
tgcttaacacatgcaagtcgaacgtgaaagtccttcggggcgagtaaagtggcgcacgggtgagtaacgcgtggataatctacccttaagatggggataacggctggaaacggtcgctaataccgaatacgctcccgattttatcattggggggaaagatggcctctgcttgcaagctatcgcttaaggatgagtccgcgtcccattagctagttggcggggtaacggcccaccaaggcaacgatgggtagccggtctgagaggatgaccggccacactggaactggaacacggtccagactcctacgggaggcagcagtggggaatattgcgcaatgggcgaaagcctgacgcagcgacgccgcgtgagggatgaaggttctcggatcgtaaacctctgtcaggggggaagaaaccccctcgtgtgaataatgcgagggcttgacggtacccccaaaggaagcaccggctaactccgtgccagcagccgcggtaatacggagggtgcaagcgttaatcggaatcactgggcgtaaagcgcacgtaggcggcttggtaagtcaggggtgaaatcccacagcccaactgtggaactgcctttgatactgccaggcttgagtaccggagagggtggcggaattccaggtgtaggagtgaaatccgtagatatctggaggaacaccggtggcgaaggcggccacctggacggtaactgacgctgaggtgcgaaagcgtgggtagcaaacaggattagataccctggtagtccacgctgtaaacgatgggtgctgggtgctgggatgtatgtctcggtgccgtagctaacgcgataagcaccccgcctggggagtacggtcgcaaggctgaaactcaaagaaattgacgggggcccgcacaagcggtggagtatgtggtttaattcgatgcaacgcgaagaaccttacccaggcttgacatctagggaacccttcggaaatgaaggggtgcccttcggggagccctaagacaggtgctgcatggctgtcgtcagctcgtgccgtgaggtgttgggttaagtcccgcaacgagcgcaacccctatcttcagttgccagcaggtaaggctgggcactctggagagaccgccccggtcaacggggaggaaggtggggacgacgtcaagtcatcatggcccttacgcctggggctacacacgtactacaatggcgcgcacaaagggtagcgagaccgcgaggtggagccaatcccaaaaaacgcgtcccagtccggattggagtctgcaactcgactccatgaagtcggaatcgctagtaattcgagatcagcatgctcgggtgaatgcgttcccgggccttgtacacaccgcccgtcacaccacgaaagtcggttttacccgaagccggtgagctaactcgcaagaggagcagccgtctacggtagggccgatgattgggg